European Patent Application EP 4 741 419 A1, published May 13, 2026. Title: 一种角蛋白CF4、制法和其药物组合物与用途. Applicant: 中国医学科学院药物研究所. The sequence listing filed with the application follows.

SEQUENCE LISTING (2 sequences)

SEQ ID NO: 1 - protein, 421 aa, unidentified
MTCGFSSVGCGFSPRTFSCASACGPRPGRCCITAAPYRGVSCYRGLCGGFGSRSLCGGFRAGSCGRSFGYRSGGVRGPSAPCITTVSVNESLLAPLNLEIDPNAQYVKQEEKEQIKSLNNRFAAFIDKVRFLEQQNKLLETKLQFYQNRKCCDSNLEPLFSGYLEALWREAECVEADSGRLASELSHVQEVLEGYKKRYEEEVTLRATAENEFVALKKDVDCAYLRKSDLEANAEALTQEVDFLRRLYEEEIRVLQAHISDTSVIVKMDNSRDLNLASIVAEIKAHYDDIASRSRAEAESWYRTKCEEIKATVVRHGETLRRTKEEINELNRLIQQLTAEIENAKCQNSKLEAAVAEAEQQGEAALNDARCKLAGLEDALQKAKQDMACLLREYQEVLNSKLGLDIEIATYRRLLEGEEQR

SEQ ID NO: 2 - DNA, 1263 bp, unidentified
  source 1..1263: mol_type = other DNA
atgacctgcggctttagcagcgtgggctgtggctttagcccgcgcacctttagctgtgcgagcgcgtgtggtcctcgtccgggtcgttgttgtattaccgcggcgccttatcgcggcgttagctgttatcgtggtttatgcggcggctttggtagccgcagcttatgtggtggctttcgcgcgggtagctgtggtcgttcatttggttatcgcagcggcggtgtgcgtggcccttcagcgccttgtattaccaccgttagcgtgaatgaaagcctgctggcgccgctgaatctggaaattgatccgaacgcgcagtatgtgaaacaggaagaaaaagaacagatcaagagcctgaacaaccgctttgcggcgtttattgataaagtgcgctttctggaacagcagaacaaactgctggaaaccaaactgcagttttatcagaaccgcaaatgctgcgatagcaacctggaaccgctgtttagcggctatctggaagcgctgtggcgcgaagcagaatgcgttgaagcggatagcggccgtttagcgagcgaactgtcacatgttcaagaagtgctggaaggctataaaaaacgctatgaagaagaggtgaccctgcgcgcgaccgcggaaaatgaatttgtggcgctgaaaaaagatgtggactgcgcgtatctgcgcaaaagcgatctggaagcgaacgcggaagcgctgacccaagaagttgattttctgcgccgcctgtatgaagaagaaattcgcgtgctgcaggcgcatattagcgataccagcgtgattgtgaaaatggataacagccgcgatctgaacctggcgagcattgtggcggaaattaaagcgcattatgatgacattgcgagccgcagccgcgcggaagcagaaagctggtatcgtaccaaatgcgaagaaattaaagcgaccgtggtgcgccatggcgaaaccttacgtcgcaccaaagaagaaattaacgaactgaaccgcctgattcagcagctgaccgcggaaattgaaaacgcgaaatgccagaacagcaaactggaagcggcggtggcggaagcggaacaacaaggcgaagcggcgttaaatgatgcgcgctgcaaactggcgggcctggaagatgcgttacaaaaagcgaaacaggatatggcgtgcctgctgcgcgaatatcaggaagtgctgaacagcaaactgggcctggatattgaaattgcgacctatcgccgcctgctggaaggcgaagaacagcgc